European Patent Application EP 4 600 349 A1, published August 13, 2025. Title: Stromal cell layer around intestinal organoids for enhancing engraftment and regenerative ability and use thereof. Applicant: 한국생명공학연구원. The sequence listing filed with the application follows.

SEQUENCE LISTING (70 sequences)

SEQ ID NO: 1 - DNA, 19 bp, synthetic construct
  source 1..19: mol_type = other DNA
gaaggtgaaggtcggagtc

SEQ ID NO: 2 - DNA, 20 bp, synthetic construct
  source 1..20: mol_type = other DNA
gaagatggtgatgggatttc

SEQ ID NO: 3 - DNA, 20 bp, synthetic construct
  source 1..20: mol_type = other DNA
ttcaatgtcccagccatgta

SEQ ID NO: 4 - DNA, 20 bp, synthetic construct
  source 1..20: mol_type = other DNA
gaaggaatagccacgctcag

SEQ ID NO: 5 - DNA, 24 bp, synthetic construct
  source 1..24: mol_type = other DNA
agaacgtgcaggaggcagaagaat

SEQ ID NO: 6 - DNA, 24 bp, synthetic construct
  source 1..24: mol_type = other DNA
ttccatttcacgcatctggcgttc

SEQ ID NO: 7 - DNA, 20 bp, synthetic construct
  source 1..20: mol_type = other DNA
cagtggctaccaggacaaca

SEQ ID NO: 8 - DNA, 20 bp, synthetic construct
  source 1..20: mol_type = other DNA
ctcagaacccctttgctcag

SEQ ID NO: 9 - DNA, 20 bp, synthetic construct
  source 1..20: mol_type = other DNA
tgcggccaaatgttattttc

SEQ ID NO: 10 - DNA, 20 bp, synthetic construct
  source 1..20: mol_type = other DNA
tgcatggtttctgacatcgt

SEQ ID NO: 11 - DNA, 20 bp, synthetic construct
  source 1..20: mol_type = other DNA
cagcccaaagtgtgtgagaa

SEQ ID NO: 12 - DNA, 20 bp, synthetic construct
  source 1..20: mol_type = other DNA
cggtcaaactgcccatactt

SEQ ID NO: 13 - DNA, 21 bp, synthetic construct
  source 1..21: mol_type = other DNA
gagcatgagggaagatgcgac

SEQ ID NO: 14 - DNA, 21 bp, synthetic construct
  source 1..21: mol_type = other DNA
tgaccacaccaactaggatga

SEQ ID NO: 15 - DNA, 20 bp, synthetic construct
  source 1..20: mol_type = other DNA
gctttccatccaggtgtcat

SEQ ID NO: 16 - DNA, 20 bp, synthetic construct
  source 1..20: mol_type = other DNA
accacgaatccatctccaac

SEQ ID NO: 17 - DNA, 20 bp, synthetic construct
  source 1..20: mol_type = other DNA
agccagatcactgctgaggt

SEQ ID NO: 18 - DNA, 20 bp, synthetic construct
  source 1..20: mol_type = other DNA
tggacaggtgttcctccttc

SEQ ID NO: 19 - DNA, 20 bp, synthetic construct
  source 1..20: mol_type = other DNA
tggcctacacaagcatctgg

SEQ ID NO: 20 - DNA, 20 bp, synthetic construct
  source 1..20: mol_type = other DNA
taactggctgctgtaacggg

SEQ ID NO: 21 - DNA, 21 bp, synthetic construct
  source 1..21: mol_type = other DNA
aaaaccccaggagcagttaat

SEQ ID NO: 22 - DNA, 20 bp, synthetic construct
  source 1..20: mol_type = other DNA
caaccctctttgcacaagct

SEQ ID NO: 23 - DNA, 20 bp, synthetic construct
  source 1..20: mol_type = other DNA
ggtaaggagaaaccgggaag

SEQ ID NO: 24 - DNA, 20 bp, synthetic construct
  source 1..20: mol_type = other DNA
gcacgtcgacctatggaaat

SEQ ID NO: 25 - DNA, 20 bp, synthetic construct
  source 1..20: mol_type = other DNA
tcctcgcctacaacctcaac

SEQ ID NO: 26 - DNA, 20 bp, synthetic construct
  source 1..20: mol_type = other DNA
gctgggacactccattctct

SEQ ID NO: 27 - DNA, 20 bp, synthetic construct
  source 1..20: mol_type = other DNA
acctttcccgtggacagagt

SEQ ID NO: 28 - DNA, 23 bp, synthetic construct
  source 1..23: mol_type = other DNA
tggacatattccctcactttgga

SEQ ID NO: 29 - DNA, 20 bp, synthetic construct
  source 1..20: mol_type = other DNA
tgacctcaacgatgcatttc

SEQ ID NO: 30 - DNA, 20 bp, synthetic construct
  source 1..20: mol_type = other DNA
ctgtcctggctcttctgctc

SEQ ID NO: 31 - DNA, 20 bp, synthetic construct
  source 1..20: mol_type = other DNA
gggcaccaaagagcatagag

SEQ ID NO: 32 - DNA, 20 bp, synthetic construct
  source 1..20: mol_type = other DNA
aaagcacacgcacgttgtag

SEQ ID NO: 33 - DNA, 20 bp, synthetic construct
  source 1..20: mol_type = other DNA
cctcctccgactgaagacag

SEQ ID NO: 34 - DNA, 20 bp, synthetic construct
  source 1..20: mol_type = other DNA
tggtctgggtacaggcctac

SEQ ID NO: 35 - DNA, 20 bp, synthetic construct
  source 1..20: mol_type = other DNA
tgctttcaacgtggagtttg

SEQ ID NO: 36 - DNA, 20 bp, synthetic construct
  source 1..20: mol_type = other DNA
ccccatatttggtgttccag

SEQ ID NO: 37 - DNA, 20 bp, synthetic construct
  source 1..20: mol_type = other DNA
tgtaggcatcgctcttctca

SEQ ID NO: 38 - DNA, 20 bp, synthetic construct
  source 1..20: mol_type = other DNA
gacaccatctacctcacccg

SEQ ID NO: 39 - DNA, 20 bp, synthetic construct
  source 1..20: mol_type = other DNA
cggatgactgcctcaatggt

SEQ ID NO: 40 - DNA, 20 bp, synthetic construct
  source 1..20: mol_type = other DNA
aaagacgctcccttctgctc

SEQ ID NO: 41 - DNA, 21 bp, synthetic construct
  source 1..21: mol_type = other DNA
cagaagactgggaacatttga

SEQ ID NO: 42 - DNA, 20 bp, synthetic construct
  source 1..20: mol_type = other DNA
cacacttgaacacgccactt

SEQ ID NO: 43 - DNA, 20 bp, synthetic construct
  source 1..20: mol_type = other DNA
cgtgaagctggtgaacttgg

SEQ ID NO: 44 - DNA, 20 bp, synthetic construct
  source 1..20: mol_type = other DNA
ggatgtactccacggctgag

SEQ ID NO: 45 - DNA, 22 bp, synthetic construct
  source 1..22: mol_type = other DNA
gagtggacttgtgccgacttca

SEQ ID NO: 46 - DNA, 22 bp, synthetic construct
  source 1..22: mol_type = other DNA
ggtggctggtgcaaagacatag

SEQ ID NO: 47 - DNA, 20 bp, synthetic construct
  source 1..20: mol_type = other DNA
gctcgagaaggatgtggtcc

SEQ ID NO: 48 - DNA, 20 bp, synthetic construct
  source 1..20: mol_type = other DNA
cgttgtgcatagtcgctgct

SEQ ID NO: 49 - DNA, 20 bp, synthetic construct
  source 1..20: mol_type = other DNA
gcagaaggcctcagcaccta

SEQ ID NO: 50 - DNA, 19 bp, synthetic construct
  source 1..19: mol_type = other DNA
aggttcccagtcgggttca

SEQ ID NO: 51 - DNA, 26 bp, synthetic construct
  source 1..26: mol_type = other DNA
tgggagcggtgaagatggaagggcac

SEQ ID NO: 52 - DNA, 26 bp, synthetic construct
  source 1..26: mol_type = other DNA
tcatgccagcgcccacgtacgacgac

SEQ ID NO: 53 - DNA, 26 bp, synthetic construct
  source 1..26: mol_type = other DNA
cgctttcatggtgtgggctaaggacg

SEQ ID NO: 54 - DNA, 26 bp, synthetic construct
  source 1..26: mol_type = other DNA
tagttggggtggtcctgcatgtgctg

SEQ ID NO: 55 - DNA, 22 bp, synthetic construct
  source 1..22: mol_type = other DNA
ctggagctggagaaggagtttc

SEQ ID NO: 56 - DNA, 24 bp, synthetic construct
  source 1..24: mol_type = other DNA
attttaacctgcctctcagagagc

SEQ ID NO: 57 - DNA, 20 bp, synthetic construct
  source 1..20: mol_type = other DNA
tgctcttcaccaactgcatc

SEQ ID NO: 58 - DNA, 20 bp, synthetic construct
  source 1..20: mol_type = other DNA
ctcaggctcaccagatcctc

SEQ ID NO: 59 - DNA, 20 bp, synthetic construct
  source 1..20: mol_type = other DNA
gggggaggttggactgtaat

SEQ ID NO: 60 - DNA, 20 bp, synthetic construct
  source 1..20: mol_type = other DNA
gaataggctcggttcccttc

SEQ ID NO: 61 - DNA, 20 bp, synthetic construct
  source 1..20: mol_type = other DNA
cccacgttttcagagttggt

SEQ ID NO: 62 - DNA, 20 bp, synthetic construct
  source 1..20: mol_type = other DNA
cggctctttcgcttactgtt

SEQ ID NO: 63 - DNA, 20 bp, synthetic construct
  source 1..20: mol_type = other DNA
cctttgcaggaaatggactc

SEQ ID NO: 64 - DNA, 20 bp, synthetic construct
  source 1..20: mol_type = other DNA
ggactcacgggtagcacaac

SEQ ID NO: 65 - DNA, 20 bp, synthetic construct
  source 1..20: mol_type = other DNA
gtgcagtcagcacaaagtgg

SEQ ID NO: 66 - DNA, 20 bp, synthetic construct
  source 1..20: mol_type = other DNA
atgcacatccggaatgggtt

SEQ ID NO: 67 - DNA, 20 bp, synthetic construct
  source 1..20: mol_type = other DNA
atctcctgtttgaccggcag

SEQ ID NO: 68 - DNA, 20 bp, synthetic construct
  source 1..20: mol_type = other DNA
gtcgtcagagtcggggtttg

SEQ ID NO: 69 - DNA, 19 bp, synthetic construct
  source 1..19: mol_type = other DNA
gtggcatcgttgaggagtg

SEQ ID NO: 70 - DNA, 19 bp, synthetic construct
  source 1..19: mol_type = other DNA
cacgtccctctcggacttg